European Patent Application EP 4 585 690 A1, published July 16, 2025. Title: Construct of self-circularization RNA. Applicant: Rznomics Inc. Application KR. The sequence listing filed with the application follows.

SEQUENCE LISTING (73 sequences)

SEQ ID NO: 1-2 - skipped (2 entries)

SEQ ID NO: 3 - DNA, 20 bp, synthetic construct
  misc_feature 1..20: note = T7 promoter
  source 1..20: mol_type = other DNA
taatacgactcactataggg

SEQ ID NO: 4 - DNA, 151 bp, synthetic construct
  misc_feature 1..151: note = AS 150
  source 1..151: mol_type = other DNA
cggcggccagcatggagaactgccatggctcagccaggtagtactgtgggtactcgaagtggctgcgtaccacacccgtcgcattggagaagggcacgtagaagttagggccttctgtgccattcatggctgtggcccttgtggctgaccc

SEQ ID NO: 5 - skipped

SEQ ID NO: 6 - DNA, 387 bp, synthetic construct
  misc_feature 1..387: note = Trans splicing ribozyme
  source 1..387: mol_type = other DNA
aaaagttatcaggcatgcacctggtagctagtctttaaaccaatagattgcatcggtttaaaaggcaagaccgtcaaattgcgggaaaggggtcaacagccgttcagtaccaagtctcaggggaaactttgagatggccttgcaaagggtatggtaataagctgacggacatggtcctaaccacgcagccaagtcctaagtcaacagatcttctgttgatatggatgcagttcacagactaaatgtcggtcggggaagatgtattcttctcataagatatagtcggacctctccttaatgggagctagcggatgaagtgatgcaacactggagccgctgggaactaatttgtatgcgaaagtatattgattagttttggagtactcg

SEQ ID NO: 7 - DNA, 463 bp, synthetic construct
  misc_feature 1..463: note = EMCV IRES
  source 1..463: mol_type = other DNA
gagggcccggaaacctggccctgtcttcttgacgagcattcctaggggtctttcccctctcgccaaaggaatgcaaggtctgttgaatgtcgtgaaggaagcagttcctctggaagcttcttgaagacaaacaacgtctgtagcgaccctttgcaggcagcggaaccccccacctggcgacaggtgcctctgcggccaaaagccacgtgtataagatacacctgcaaaggcggcacaaccccagtgccacgttgtgagttggatagttgtggaaagagtcaaatggctctcctcaagcgtattcaacaaggggctgaaggatgcccagaaggtaccccattgtatgggatctgatctggggcctcggtgcacatgctttacatgtgtttagtcgaggttaaaaaaacgtctaggccccccgaaccacggggacgtggttttcctttgaaaaacacgatgataa

SEQ ID NO: 8 - DNA, 558 bp, synthetic construct
  misc_feature 1..558: note = Gaussia Luciferase
  source 1..558: mol_type = other DNA
atgggagtcaaagttctgtttgccctgatctgcatcgctgtggccgaggccaagcccaccgagaacaacgaagacttcaacatcgtggccgtggccagcaacttcgcgaccacggatctcgatgctgaccgcgggaagttgcccggcaagaagctgccgctggaggtgctcaaagagatggaagccaatgcccggaaagctggctgcaccaggggctgtctgatctgcctgtcccacatcaagtgcacgcccaagatgaagaagttcatcccaggacgctgccacacctacgaaggcgacaaagagtccgcacagggcggcataggcgaggcgatcgtcgacattcctgagattcctgggttcaaggacttggagcccatggagcagttcatcgcacaggtcgatctgtgtgtggactgcacaactggctgcctcaaagggcttgccaacgtgcagtgttctgacctgctcaagaagtggctgccgcaacgctgtgcgacctttgccagcaagatccagggccaggtggacaagatcaagggggccggtggtgactaa

SEQ ID NO: 9 - DNA, 150 bp, synthetic construct
  misc_feature 1..150: note = Antisense Binding Sequecne
  source 1..150: mol_type = other DNA
gggtcagccacaagggccacagccatgaatggcacagaaggccctaacttctacgtgcccttctccaatgcgacgggtgtggtacgcagccacttcgagtacccacagtactacctggctgagccatggcagttctccatgctggccgcc

SEQ ID NO: 10 - DNA, 1908 bp, synthetic construct
  misc_feature 1..1908: note = DNA template encoding self-circularizaion RNA of the example 1
  source 1..1908: mol_type = other DNA
gggattcgaacatcgattaatacgactcactataggggcatcgattgaattgtcgacgaattcggcggccagcatggagaactgccatggctcagccaggtagtactgtgggtactcgaagtggctgcgtaccacacccgtcgcattggagaagggcacgtagaagttagggccttctgtgccattcatggctgtggcccttgtggctgacccgaattccgtactccgcccaaaaaagttatcaggcatgcacctggtagctagtctttaaaccaatagattgcatcggtttaaaaggcaagaccgtcaaattgcgggaaaggggtcaacagccgttcagtaccaagtctcaggggaaactttgagatggccttgcaaagggtatggtaataagctgacggacatggtcctaaccacgcagccaagtcctaagtcaacagatcttctgttgatatggatgcagttcacagactaaatgtcggtcggggaagatgtattcttctcataagatatagtcggacctctccttaatgggagctagcggatgaagtgatgcaacactggagccgctgggaactaatttgtatgcgaaagtatattgattagttttggagtactcgcgagtacgcttaagaaaaaaaaaagagggcccggaaacctggccctgtcttcttgacgagcattcctaggggtctttcccctctcgccaaaggaatgcaaggtctgttgaatgtcgtgaaggaagcagttcctctggaagcttcttgaagacaaacaacgtctgtagcgaccctttgcaggcagcggaaccccccacctggcgacaggtgcctctgcggccaaaagccacgtgtataagatacacctgcaaaggcggcacaaccccagtgccacgttgtgagttggatagttgtggaaagagtcaaatggctctcctcaagcgtattcaacaaggggctgaaggatgcccagaaggtaccccattgtatgggatctgatctggggcctcggtgcacatgctttacatgtgtttagtcgaggttaaaaaaacgtctaggccccccgaaccacggggacgtggttttcctttgaaaaacacgatgataagcttgccacaacccttaagaccggtatgggagtcaaagttctgtttgccctgatctgcatcgctgtggccgaggccaagcccaccgagaacaacgaagacttcaacatcgtggccgtggccagcaacttcgcgaccacggatctcgatgctgaccgcgggaagttgcccggcaagaagctgccgctggaggtgctcaaagagatggaagccaatgcccggaaagctggctgcaccaggggctgtctgatctgcctgtcccacatcaagtgcacgcccaagatgaagaagttcatcccaggacgctgccacacctacgaaggcgacaaagagtccgcacagggcggcataggcgaggcgatcgtcgacattcctgagattcctgggttcaaggacttggagcccatggagcagttcatcgcacaggtcgatctgtgtgtggactgcacaactggctgcctcaaagggcttgccaacgtgcagtgttctgacctgctcaagaagtggctgccgcaacgctgtgcgacctttgccagcaagatccagggccaggtggacaagatcaagggggccggtggtgactaaaaaaaaaaaaaccggtttgggtgggagcagccacgggtcagccacaagggccacagccatgaatggcacagaaggccctaacttctacgtgcccttctccaatgcgacgggtgtggtacgcagccacttcgagtacccacagtactacctggctgagccatggcagttctccatgctggccgccaagcttgcctcgagcagcgctgctcgagagatct

SEQ ID NO: 11 - DNA, 56 bp, synthetic construct
  misc_feature 1..56: note = T7 Circular Forward primer
  source 1..56: mol_type = other DNA
gggattcgaacatcgattaatacgactcactataggggcatcgattgaattgtcga

SEQ ID NO: 12 - DNA, 34 bp, synthetic construct
  misc_feature 1..34: note = T7 Circular Reverse primer
  source 1..34: mol_type = other DNA
agatctctcgagcagcgctgctcgaggcaagctt

SEQ ID NO: 13 - DNA, 21 bp, synthetic construct
  misc_feature 1..21: note = Circular STS Forward primer of the example 2-2
  source 1..21: mol_type = other DNA
ccctgagtggctgagctcagg

SEQ ID NO: 14 - DNA, 23 bp, synthetic construct
  misc_feature 1..23: note = Circular STS Reverse primer of the example 2-2
  source 1..23: mol_type = other DNA
cagcaagcatactaaattgccag

SEQ ID NO: 15 - DNA, 25 bp, synthetic construct
  misc_feature 1..25: note = Circular STS Forward primer of the example 3
  source 1..25: mol_type = other DNA
caaggacttggagcccatggagcag

SEQ ID NO: 16 - DNA, 23 bp, synthetic construct
  misc_feature 1..23: note = Circular STS Reverse primer 2 of the example 3
  source 1..23: mol_type = other DNA
tgtgccgcctttgcaggtgtatc

SEQ ID NO: 17 - DNA, 50 bp, synthetic construct
  misc_feature 1..50: note = AS50
  source 1..50: mol_type = other DNA
aagttagggccttctgtgccattcatggctgtggcccttgtggctgaccc

SEQ ID NO: 18 - DNA, 100 bp, synthetic construct
  misc_feature 1..100: note = AS100
  source 1..100: mol_type = other DNA
actcgaagtggctgcgtaccacacccgtcgcattggagaagggcacgtagaagttagggccttctgtgccattcatggctgtggcccttgtggctgaccc

SEQ ID NO: 19 - DNA, 150 bp, synthetic construct
  misc_feature 1..150: note = AS150
  source 1..150: mol_type = other DNA
ggcggccagcatggagaactgccatggctcagccaggtagtactgtgggtactcgaagtggctgcgtaccacacccgtcgcattggagaagggcacgtagaagttagggccttctgtgccattcatggctgtggcccttgtggctgaccc

SEQ ID NO: 20 - DNA, 200 bp, synthetic construct
  misc_feature 1..200: note = AS200
  source 1..200: mol_type = other DNA
agcgtgaggaagttgatggggaagcccagcacgatcagcagaaacatgtaggcggccagcatggagaactgccatggctcagccaggtagtactgtgggtactcgaagtggctgcgtaccacacccgtcgcattggagaagggcacgtagaagttagggccttctgtgccattcatggctgtggcccttgtggctgaccc

SEQ ID NO: 21 - DNA, 250 bp, synthetic construct
  misc_feature 1..250: note = AS250
  source 1..250: mol_type = other DNA
ggatgtagttgagaggcgtgcgcagcttcttgtgctggacggtgacgtagagcgtgaggaagttgatggggaagcccagcacgatcagcagaaacatgtaggcggccagcatggagaactgccatggctcagccaggtagtactgtgggtactcgaagtggctgcgtaccacacccgtcgcattggagaagggcacgtagaagttagggccttctgtgccattcatggctgtggcccttgtggctgaccc

SEQ ID NO: 22 - DNA, 300 bp, synthetic construct
  misc_feature 1..300: note = AS300
  source 1..300: mol_type = other DNA
ggtgaagccacctaggaccatgaagaggtcagccacggctaggttgagcaggatgtagttgagaggcgtgcgcagcttcttgtgctggacggtgacgtagagcgtgaggaagttgatggggaagcccagcacgatcagcagaaacatgtaggcggccagcatggagaactgccatggctcagccaggtagtactgtgggtactcgaagtggctgcgtaccacacccgtcgcattggagaagggcacgtagaagttagggccttctgtgccattcatggctgtggcccttgtggctgaccc

SEQ ID NO: 23 - DNA, 10 bp, synthetic construct
  misc_feature 1..10: note = A10
  source 1..10: mol_type = other DNA
aaaaaaaaaa

SEQ ID NO: 24 - DNA, 30 bp, synthetic construct
  misc_feature 1..30: note = A30
  source 1..30: mol_type = other DNA
aaaaaaaaaaaaaaaaaaaaaaaaaaaaaa

SEQ ID NO: 25 - DNA, 39 bp, synthetic construct
  misc_feature 1..39: note = A50
  source 1..39: mol_type = other DNA
aaaaaaaaaaaaaaaaaaaaaaaaaaaaaaaaaaaaaaa

SEQ ID NO: 26 - DNA, 35 bp, synthetic construct
  misc_feature 1..35: note = Control spacer 1
  source 1..35: mol_type = other DNA
ggtagtggtgctactaacttcagcctgctgaagca

SEQ ID NO: 27 - DNA, 34 bp, synthetic construct
  misc_feature 1..34: note = Control spacer 2
  source 1..34: mol_type = other DNA
ggtagtaaactactaactacaacctgctgaagca

SEQ ID NO: 28 - skipped

SEQ ID NO: 29 - DNA, 1522 bp, synthetic construct
  misc_feature 1..1522: note = DNA template encoding self-circularizaion RNA of the example 7
  source 1..1522: mol_type = other DNA
gggattcgaacatcgattaatacgactcactataggggcccaaaaaagttatcaggcatgcacctggtagctagtctttaaaccaatagattgcatcggtttaaaaggcaagaccgtcaaattgcgggaaaggggtcaacagccgttcagtaccaagtctcaggggaaactttgagatggccttgcaaagggtatggtaataagctgacggacatggtcctaaccacgcagccaagtcctaagtcaacagatcttctgttgatatggatgcagttcacagactaaatgtcggtcggggaagatgtattcttctcataagatatagtcggacctctccttaatgggagctagcggatgaagtgatgcaacactggagccgctgggaactaatttgtatgcgaaagtatattgattagttttggagtactcgcgagtacgcttaagaaaaaaaaaagagggcccggaaacctggccctgtcttcttgacgagcattcctaggggtctttcccctctcgccaaaggaatgcaaggtctgttgaatgtcgtgaaggaagcagttcctctggaagcttcttgaagacaaacaacgtctgtagcgaccctttgcaggcagcggaaccccccacctggcgacaggtgcctctgcggccaaaagccacgtgtataagatacacctgcaaaggcggcacaaccccagtgccacgttgtgagttggatagttgtggaaagagtcaaatggctctcctcaagcgtattcaacaaggggctgaaggatgcccagaaggtaccccattgtatgggatctgatctggggcctcggtgcacatgctttacatgtgtttagtcgaggttaaaaaaacgtctaggccccccgaaccacggggacgtggttttcctttgaaaaacacgatgataagcttgccacaacccttaagaccggtatgggagtcaaagttctgtttgccctgatctgcatcgctgtggccgaggccaagcccaccgagaacaacgaagacttcaacatcgtggccgtggccagcaacttcgcgaccacggatctcgatgctgaccgcgggaagttgcccggcaagaagctgccgctggaggtgctcaaagagatggaagccaatgcccggaaagctggctgcaccaggggctgtctgatctgcctgtcccacatcaagtgcacgcccaagatgaagaagttcatcccaggacgctgccacacctacgaaggcgacaaagagtccgcacagggcggcataggcgaggcgatcgtcgacattcctgagattcctgggttcaaggacttggagcccatggagcagttcatcgcacaggtcgatctgtgtgtggactgcacaactggctgcctcaaagggcttgccaacgtgcagtgttctgacctgctcaagaagtggctgccgcaacgctgtgcgacctttgccagcaagatccagggccaggtggacaagatcaagggggccggtggtgactaaaaaaaaaaaaaccggtttgggt

SEQ ID NO: 30-46 - skipped (17 entries)

SEQ ID NO: 47 - RNA, 17 nt, synthetic construct
  misc_feature 1..17: note = Fig 13_P1&P10_5' end
  source 1..17: mol_type = other RNA
gggcgtactccgcccaa

SEQ ID NO: 48 - skipped

SEQ ID NO: 49 - RNA, 17 nt, synthetic construct
  misc_feature 1..17: note = Fig 13_P1&P10+AS150_5' end
  source 1..17: mol_type = other RNA
gggcgtactccgcccaa

SEQ ID NO: 50-58 - skipped (9 entries)

SEQ ID NO: 59 - RNA, 17 nt, synthetic construct
  misc_feature 1..17: note = Fig 21a_P1&P10_P1&P10 helix_5'end
  source 1..17: mol_type = other RNA
aacccgcctcatgcggg

SEQ ID NO: 60-64 - skipped (5 entries)

SEQ ID NO: 65 - RNA, 11 nt, synthetic construct
  misc_feature 1..11: note = Fig 21a_P1 Bulge+AS150_P1 helix_3'end
  source 1..11: mol_type = other RNA
ttgggtagcag

SEQ ID NO: 66 - RNA, 12 nt, synthetic construct
  misc_feature 1..12: note = Fig 21a_P1 Bulge+AS150_P1 helix_5'end
  source 1..12: mol_type = other RNA
aacccgcttaag

SEQ ID NO: 67 - RNA, 15 nt, synthetic construct
  misc_feature 1..15: note = Fig 21a_P1 Extention&Bulge+AS150_P1 helix_3'end
  source 1..15: mol_type = other RNA
ttgggtcctagcagc

SEQ ID NO: 68 - RNA, 15 nt, synthetic construct
  misc_feature 1..15: note = Fig 21a_P1 Extention&Bulge+AS150_P1 helix_5'end
  source 1..15: mol_type = other RNA
aacccggggcttaag

SEQ ID NO: 69 - DNA, 46 bp, synthetic construct
  misc_feature 1..46: note = T7 No P10 F primer (P1)
  source 1..46: mol_type = other DNA
ataatacgactcactataggggcccaaaaaagttatcaggcatgca

SEQ ID NO: 70 - DNA, 35 bp, synthetic construct
  misc_feature 1..35: note = No P10 R primer (P1)
  source 1..35: mol_type = other DNA
acccaaaccggtttttttttttttagtcaccaccg

SEQ ID NO: 71 - DNA, 38 bp, synthetic construct
  misc_feature 1..38: note = P1 Extension R primer (P1)
  source 1..38: mol_type = other DNA
aggacccaaaccggtttttttttttttagtcaccaccg

SEQ ID NO: 72 - DNA, 34 bp, synthetic construct; identical to SEQ ID NO: 12
  misc_feature 1..34: note = Circular RNA R primer (comprising an AS150)
  source 1..34: mol_type = other DNA

SEQ ID NO: 73 - DNA, 52 bp, synthetic construct
  misc_feature 1..52: note = Fig 22d
  source 1..52: mol_type = other DNA
actaaaaaaaaaaaaaccggtttgggtcgagtacgcttaagaaaaaaaaaag